European Patent Application EP 4 494 460 A1, published January 22, 2025. Title: SELF-INCOMPATIBLE DIHAPLOID POTATO LINE AND PRODUCTION METHOD THEREFOR, AND HYBRID POTATO AND SEED PRODUCTION METHOD THEREFOR. Applicant: AGRICULTURAL GENOMICS INSTITUTE AT SHENZHEN, CHINESE ACADEMY OF AGRICULTURAL SCIENCES (SHENZHEN BRANCH, GUANGDONG LABORATORY FOR LINGNAN MODERN AGRICULTURE). Application EP. The sequence listing filed with the application follows.

SEQUENCE LISTING (16 sequences)

SEQ ID NO: 1 - DNA, 20 bp, synthetic construct
  source 1..20: mol_type = other DNA
tacaaatattcagcgaaggg

SEQ ID NO: 2 - DNA, 22 bp, synthetic construct
  source 1..22: mol_type = other DNA
gctcaattgtcttcttcaatcc

SEQ ID NO: 3 - DNA, 20 bp, synthetic construct
  source 1..20: mol_type = other DNA
tcctccatctcagattcact

SEQ ID NO: 4 - DNA, 20 bp, synthetic construct
  source 1..20: mol_type = other DNA
gggtacgattgtgaacatct

SEQ ID NO: 5 - DNA, 20 bp, synthetic construct
  source 1..20: mol_type = other DNA
ctataatttgggcacgtgat

SEQ ID NO: 6 - DNA, 20 bp, synthetic construct
  source 1..20: mol_type = other DNA
ctagttgcattcagccttct

SEQ ID NO: 7 - DNA, 21 bp, synthetic construct
  source 1..21: mol_type = other DNA
cagagacaggaacagaaaatg

SEQ ID NO: 8 - DNA, 20 bp, synthetic construct
  source 1..20: mol_type = other DNA
tgaagggactaatttggcta

SEQ ID NO: 9 - DNA, 20 bp, synthetic construct
  source 1..20: mol_type = other DNA
gggatcatttcgatctttct

SEQ ID NO: 10 - DNA, 20 bp, synthetic construct
  source 1..20: mol_type = other DNA
gtaaattggaaatccctcct

SEQ ID NO: 11 - DNA, 20 bp, synthetic construct
  source 1..20: mol_type = other DNA
tgaccctttggatgaaatac

SEQ ID NO: 12 - DNA, 20 bp, synthetic construct
  source 1..20: mol_type = other DNA
caccttatcaaacgaagctc

SEQ ID NO: 13 - DNA, 27 bp, synthetic construct
  source 1..27: mol_type = other DNA
gaagaaaggaaatgaagtgagttgttc

SEQ ID NO: 14 - DNA, 29 bp, synthetic construct
  source 1..29: mol_type = other DNA
gaataataacttatttcttgatgggattg

SEQ ID NO: 15 - DNA, 22 bp, synthetic construct
  source 1..22: mol_type = other DNA
cgtcggattcagcagcagagtt

SEQ ID NO: 16 - DNA, 29 bp, synthetic construct
  source 1..29: mol_type = other DNA
aagcgaattacaagcctgtttagattgac